European Patent Application EP 4 591 871 A1, published July 30, 2025. Title: Anti-obesity agent having intestinal bacteria as active ingredient, and method for manufacturing same. Applicant: Kabushiki Kaisha Yakult Honsha. Application IB PCT/JP2023/030711, filed August 25, 2023. The sequence listing filed with the application follows.

SEQUENCE LISTING (6 sequences)

SEQ ID NO: 1 - RNA, 20 nt, Synthetic construct
  source 1..20: mol_type = other RNA
gggcgatcttgacaggaaag

SEQ ID NO: 2 - RNA, 25 nt, Synthetic construct
  source 1..25: mol_type = other RNA
cccatcattaaggaattcatgtcat

SEQ ID NO: 3 - RNA, 20 nt, Synthetic construct
  source 1..20: mol_type = other RNA
cagcacgtgaaggtggggac

SEQ ID NO: 4 - RNA, 20 nt, Synthetic construct
  source 1..20: mol_type = other RNA
ccttgcggttggcttcagat

SEQ ID NO: 5 - RNA, 20 nt, Synthetic construct
  source 1..20: mol_type = other RNA
gaaagttagcgacggatcct

SEQ ID NO: 6 - RNA, 20 nt, Synthetic construct
  source 1..20: mol_type = other RNA
gctagagtgcccaccttgac